European Patent Application EP 4 458 845 A1, published November 6, 2024. Title: RECOMBINANT PROTEIN FOR PREVENTING OR TREATING ULCERATIVE COLITIS, AND COMPOSITION FOR PREVENTING OR TREATING ULCERATIVE COLITIS COMPRISING SAME. Applicant: NEXEL CO., LTD. Application EP. The sequence listing filed with the application follows.

SEQUENCE LISTING (4 sequences)

SEQ ID NO: 1 - protein, 202 aa, Artificial Sequence
LDICSKNPCHNGGLCEEISQEVRGDVFPSYTCTCLKGYAGNHCETKCVEPLGMENGNIANSQIAASSVRVTFLGLQHWVPELARLNRAGMVNAWTPSSNDDNPWIQVNLLRRMWVTGVVTQGASRLASHEYLKAFKVAYSLNGHEFDFIHDVNKKHKEFVGNWNKNAVHVNLFETPVEAQYVRLYPTSCHTACTLRFELLGC

SEQ ID NO: 2 - DNA, 609 bp, Artificial Sequence
  source 1..609: mol_type = other DNA
ctggatatctgcagcaaaaacccgtgccacaacggtggcctgtgcgaggaaattagccaagaggtgcgtggtgacgttttcccgagctacacctgcacctgcctgaagggctatgcgggtaaccactgcgagaccaaatgcgtggaaccgctgggcatggagaacggtaacatcgcgaacagccagattgcggcgagcagcgtgcgtgttacctttctgggcctgcaacactgggttccggaactggcgcgtctgaaccgtgcgggtatggttaacgcgtggaccccgagcagcaacgacgataacccgtggatccaggtgaacctgctgcgtcgtatgtgggttaccggcgtggttacccagggtgcgagccgtctggcgagccacgagtacctgaaggcgttcaaagttgcgtatagcctgaacggccacgaattcgactttattcacgatgtgaacaagaaacacaaggagttcgttggtaactggaacaaaaacgcggtgcacgttaacctgtttgagaccccggtggaagcgcagtacgttcgtctgtatccgaccagctgccacaccgcgtgcaccctgcgttttgaactgctgggttgctaa

SEQ ID NO: 3 - protein, 202 aa, Artificial Sequence
LDICSKNPCHNGGLCEEISQEVRGDVFPSYTCTCLKGYAGNHCETKCVEPLGLENGNIANSQIAASSVRVTFLGLQHWVPELARLNRAGMVNAWTPSSNDDNPWIQVNLLRRMWVTGVVTQGASRLASHEYLKAFKVAYSLNGHEFDFIHDVNKKHKEFVGNWNKNAVHVNLFETPVEAQYVRLYPTSCHTACTLRFELLGC

SEQ ID NO: 4 - DNA, 609 bp, Artificial Sequence
  source 1..609: mol_type = other DNA
ctggatatctgcagcaaaaacccgtgccacaacggtggcctgtgcgaggaaattagccaagaggtgcgtggtgacgttttcccgagctacacctgcacctgcctgaagggctatgcgggtaaccactgcgagaccaaatgcgtggaaccgctgggcctggagaacggtaacatcgcgaacagccagattgcggcgagcagcgtgcgtgttacctttctgggcctgcaacactgggttccggaactggcgcgtctgaaccgtgcgggtatggttaacgcgtggaccccgagcagcaacgacgataacccgtggatccaggtgaacctgctgcgtcgtatgtgggttaccggcgtggttacccagggtgcgagccgtctggcgagccacgagtacctgaaggcgttcaaagttgcgtatagcctgaacggccacgaattcgactttattcacgatgtgaacaagaaacacaaggagttcgttggtaactggaacaaaaacgcggtgcacgttaacctgtttgagaccccggtggaagcgcagtacgttcgtctgtatccgaccagctgccacaccgcgtgcaccctgcgttttgaactgctgggttgctaa